European Patent Application EP 4 144 413 A1, published March 8, 2023. Title: Composition for preventing or improving low bone strength. Applicant: AJINOMOTO CO., INC. The sequence listing filed with the application follows.

SEQUENCE LISTING (16 sequences)

SEQ ID NO: 1 - DNA, 25 bp, Artificial Sequence
  primer
acggtatcactatttaggacctgtg

SEQ ID NO: 2 - DNA, 24 bp, Artificial Sequence
  primer
actttattttggagctgctgtgac

SEQ ID NO: 3 - DNA, 21 bp, Artificial Sequence
  primer
tggagagcaccaagacagaca

SEQ ID NO: 4 - DNA, 19 bp, Artificial Sequence
  primer
tgccggagtcgacaatgat

SEQ ID NO: 5 - DNA, 23 bp, Artificial Sequence
  primer
gctggtggaaaacatcattgaca

SEQ ID NO: 6 - DNA, 19 bp, Artificial Sequence
  primer
catcggggtggctgccttt

SEQ ID NO: 7 - DNA, 22 bp, Artificial Sequence
  primer
ctggagatcacttagtccacca

SEQ ID NO: 8 - DNA, 23 bp, Artificial Sequence
  primer
gtcggaagatatgccttcacttt

SEQ ID NO: 9 - DNA, 20 bp, Artificial Sequence
  primer
aacgccacttgtccctctaa

SEQ ID NO: 10 - DNA, 20 bp, Artificial Sequence
  primer
gtggagcgatttgtctggtt

SEQ ID NO: 11 - DNA, 19 bp, Artificial Sequence
  primer
gccatggattgcacatttg

SEQ ID NO: 12 - DNA, 19 bp, Artificial Sequence
  primer
tcaggagagttggcacctg

SEQ ID NO: 13 - DNA, 20 bp, Artificial Sequence
  primer
ccagcatgatcctcttggca

SEQ ID NO: 14 - DNA, 20 bp, Artificial Sequence
  primer
tgagaggccagttgtgtgac

SEQ ID NO: 15 - DNA, 20 bp, Artificial Sequence
  primer
cgctgatgcactgcctatga

SEQ ID NO: 16 - DNA, 20 bp, Artificial Sequence
  primer
cgagtggtcttccatcacgg